European Patent Application EP 4 202 054 A1, published June 28, 2023. Title: Method for producing modified protein and method for producing property-modified protein material. Applicant: Amano Enzyme Inc. The sequence listing filed with the application follows.

SEQUENCE LISTING (1 sequence)

SEQ ID NO: 1 - protein, 312 aa, Streptomyces griseus
MRRIAGLLLAPLLLLTAVACGSDDKASDSASSKNGVPAITAGAEFGEKPTLSKGEGDPPKELKTDVISEGDGAKLKNGDAIQVNYLGQAWDSTKPFDNSFDRKQPFDLTLGAGMVIQGWDKGLVGQKVGSRVELVIPPELGYGEQGQGDIKPNATLVFVVDILKATQIPASAKGTEVAQDNVDLPKVGVKTDGKAPTVTIPKSDPPKKLVSNYVLESDGEVVKESDSVVVNYVGMIWKGAKEFDNTYSTGKTQTFPLSQVTLKGLKNGLVDKKVGSRVLLVIPPDQAFGDQQQQAIPKNSTLVFAVDILAKV